European Patent Application EP 4 792 826 A1, published August 19, 2026. Title: NGF-FC FUSION PROTEIN FORMULATION AND USE THEREOF. Applicant: STAIDSON (BEIJING) BIOPHARMACEUTICALS CO., LTD. The sequence listing filed with the application follows.

SEQUENCE LISTING (4 sequences)

SEQ ID NO: 1 - protein, 360 aa, synthetic construct
SSSHPIFHRGEESVCDSVSVWVGDKTTATDIKGKEVMVLGEVNINNSVFKQYFFETKCRDPNPVDSGCRGIDSKHWNSYCTTTHTFVKALTMDGKQAAWRFIRIDTACVCVLSRKAVRGGGGSGGGGSGGGGSDKTHTCPPCPAPEAAGGPSVFLFPPKPKDTLMISRTPEVTCVVVDVSHEDPEVKFNWYVDGVEVHNAKTKPREEQYNSTYRVVSVLTVLHQDWLNGKEYKCKVSNKALPASIEKTISKAKGQPREPQVYTLPPSREEMTKNQVSLTCLVKGFYPSDIAVEWESNGQPENNYKTTPPVLDSDGSFFLYSKLTVDKSRWQQGNVFSCSVMHEALHNHYTQKSLSLSPGK

SEQ ID NO: 2 - protein, 118 aa, synthetic construct
SSSHPIFHRGEESVCDSVSVWVGDKTTATDIKGKEVMVLGEVNINNSVFKQYFFETKCRDPNPVDSGCRGIDSKHWNSYCTTTHTFVKALTMDGKQAAWRFIRIDTACVCVLSRKAVR

SEQ ID NO: 3 - protein, 15 aa, synthetic construct
GGGGSGGGGSGGGGS

SEQ ID NO: 4 - protein, 227 aa, synthetic construct
DKTHTCPPCPAPEAAGGPSVFLFPPKPKDTLMISRTPEVTCVVVDVSHEDPEVKFNWYVDGVEVHNAKTKPREEQYNSTYRVVSVLTVLHQDWLNGKEYKCKVSNKALPASIEKTISKAKGQPREPQVYTLPPSREEMTKNQVSLTCLVKGFYPSDIAVEWESNGQPENNYKTTPPVLDSDGSFFLYSKLTVDKSRWQQGNVFSCSVMHEALHNHYTQKSLSLSPGK